European Patent Specification EP 3 788 149 B1, published August 27, 2025. Title: A Method For Optimizing Antibody Expression. Applicant: Ambrx, Inc. The sequence listing filed with the application follows.

SEQUENCE LISTING (18 sequences)

SEQ ID NO: 1 - protein, 23 aa, E. Coli
MKKNIAFLLASMFVFSIATNAYA

SEQ ID NO: 2 - protein, 110 aa, E. Coli
QAVVTQEPSLTVSPGGTVTLTCRSSTGAVTTSNYANWVQQKPGQAPRGLIGGTNKRAPGTPARFSGSLLGGKAALTLSGAQPEDEAEYYCALWYSNLWVFGGGTKLTVLG

SEQ ID NO: 3 - protein, 107 aa, E. Coli [sequence omitted]

SEQ ID NO: 4 - protein, 125 aa, E. Coli
EVQLVESGGGLVQPGGSLRLSCAASGFTFNTYAMNWVRQAPGKGLEWVARIRSKYNNYATYYADSVKDRFTISRDDSKNILYLQMNSLKTEDTAVYYCVRHGNFGNSYVSWFAYWGQGTLVTVSS

SEQ ID NO: 5 - protein, 103 aa, E. Coli
  pAcF (16)..(16): Unnatural amino acid
ASTKGPSVFPLAPSSXSTSGGTAALGCLVKDYFPEPVTVSWNSGALTSGVHTFPAVLQSSGLYSLSSVVTVPSSSLGTQTYICNVNHKPSNTKVDKKVEPKSC

SEQ ID NO: 6 - DNA, 69 bp, E. Coli
atgaaaaagaatatcgcatttcttcttgcatctatgttcgttttttctattgctacaaacgcgtacgct

SEQ ID NO: 7 - DNA, 330 bp, E.Coli
caggctgtggtgactcaggagccctcactgactgtgtccccaggagggacagtcactctcacctgtcgctccagcactggagctgtcaccactagtaattatgccaactgggtccagcagaagcctggccaagcccccaggggactgattggtgggacaaacaagagagctcccgggacacctgcccggttctcaggctccctccttgggggcaaagctgccctgaccctttcgggtgcgcagcctgaggatgaggctgagtattactgcgctctctggtatagtaatctgtgggtgttcggcggagggaccaagttgaccgtcctcgga

SEQ ID NO: 8 - DNA, 321 bp, E.Coli
cgtacggtggctgcaccatctgtcttcatcttcccgccatctgatgagcagttgaaatctggaactgcctctgttgtgtgcctgctgaataacttctatcccagagaggccaaagtacagtggaaggtggataacgccctccaatcgggtaactcccaggagagtgtcacagagcaggacagcaaggacagcacctacagcctcagcagcaccctgacgctgagcaaagcagactacgagaaacacaaagtctacgcctgcgaagtcacccatcagggcctgagctcgcccgtcacaaagagcttcaacaggggagagtgt

SEQ ID NO: 9 - DNA, 32 bp, E. Coli
tctggggataagaattcggttgaggtgatttt

SEQ ID NO: 10 - DNA, 375 bp, E. Coli
gaggtgcagctggtggagtctgggggaggcttggtccagcctggagggtccctgagactctcctgtgcagcctctggattcaccttcaatacctacgcaatgaactgggtccgccaggctccagggaaggggctggagtgggttgctcgtattagaagcaaatataacaattacgccacatattacgccgattctgtgaaagacagattcaccatctcaagagatgattcaaagaacattctgtatctgcaaatgaacagcctgaaaaccgaggacacggccgtgtattactgtgttagacatgggaatttcggcaactcttatgtcagttggtttgcctactggggccaaggtaccctggtcaccgtctcgagt

SEQ ID NO: 11 - DNA, 309 bp, E. Coli
gctagcaccaagggcccatcggtcttccccctggcaccctcctcctagagcacctctgggggcacagcggccctgggctgcctggtcaaggactacttccccgaaccggtgacggtgtcgtggaactcaggcgccctgaccagcggcgtgcacaccttcccggctgtcctacagtcctcaggactctactccctcagcagcgtggtgaccgtgccctccagcagcttgggcacccagacctacatctgcaacgtgaatcacaagcccagcaacaccaaggtggacaagaaagttgagcccaaatcttgt

SEQ ID NO: 12 - DNA, 580 bp, E. Coli
aacaaactccgggaggcagcgtgatgcggcaacaatcacacggatttcccgtgaacggtctgaatgagcggattattttcagggaaagtgagtgtggtcagcgtgcaggtatatgggctatgatgtgcccggcgcttgaggctttctgcctcatgacgtgaaggtggtttgttgccgtgttgtgtggcagaaagaagatagccccgtagtaagttaattttcattaaccaccacgaggcatccctatgtctagtccacatcaggatagcctcttaccgcgctttgcgcaaggagaagaaggccatgaaactaccacgaagttcccttgtctggtgtgtgttgatcgtgtgtctcacactgttgatattcacttatctgacacgaaaatcgctgtgcgagattcgttacagagacggacacagggaggtggcggctttcatggcttacgaatccggtaagtagcaacctggaggcgggcgcaggcccgccttttcaggactgatgctggtctgactactgaagcgcctttataaaggggctgctggttcgccggtagcccctttctccttgctgatgttgt

SEQ ID NO: 13 - DNA, 156 bp, E. Coli
atgaaactaccacgaagttcccttgtctggtgtgtgttgatcgtgtgtctcacactgttgatattcacttatctgacacgaaaatcgctgtgcgagattcgttacagagacggacacagggaggtggcggctttcatggcttacgaatccggtaag

SEQ ID NO: 14 - protein, 52 aa, E. Coli
MKLPRSSLVWCVLIVCLTLLIFTYLTRKSLCEIRYRDGHREVAAFMAYESGK

SEQ ID NO: 15 - DNA, 1199 bp, E. Coli
gattcacctcttttgtcgaatggtcgccgcggattctacttaactttgctgcccgagacagcactcatttcgcggtcatcgaaactaatttaaacaaaaagagtctgaaaatagatgataatagggcgtgtctgtatgtagatttgttcgacaacgctttatagtacccttctgataatagttaaccctggggtgagatgccccgatcctggagatatggatgaaatcactgtttaaagtaacgctgctggcgaccacaatggccgttgccctgcatgcaccaatcacttttgctgctgaagctgcaaaacctgctacagctgctgacagcaaagcagcgttcaaaaatgacgatcagaaatcagcttatgcactgggtgcctcgctgggtcgttacatggaaaactctctaaaagaacaagaaaaactgggcatcaaactggataaagatcagctgatcgctggtgttcaggatgcatttgctgataagagcaaactctccgaccaagagatcgaacagactctacaagcattcgaagctcgcgtgaagtcttctgctcaggcgaagatggaaaaagacgcggctgataacgaagcaaaaggtaaagagtaccgcgagaaatttgccaaagagaaaggtgtgaaaacctcttcaactggtctggtttatcaggtagtagaagccggtaaaggcgaagcaccgaaagacagcgatactgttgtagtgaactacaaaggtacgctgatcgacggtaaagagttcgacaactcttacacccgtggtgaaccgctttctttccgtctggacggtgttatcccgggttggacagaaggtctgaagaacatcaagaaaggcggtaagatcaaactggttattccaccagaactggcttacggcaaagcgggtgttccggggatcccaccgaattctaccctggtgtttgacgtagagctgctggatgtgaaaccagcgccgaaggctgatgcaaagccggaagctgatgcgaaagccgcagattctgctaaaaaataagcattaagaaccgccgcctgaccaggcggcggtttttttattacaggccggatataattagtgctggaaagcggaacctccgctgtattaatttagttacccgcatcattaatgagcctgccctgaaaagttaacgacaggctcctgaaaaggagtgttttttttc

SEQ ID NO: 16 - protein, 270 aa, E. Coli
MKSLFKVTLLATTMAVALHAPITFAAEAAKPATAADSKAAFKNDDQKSAYALGASLGRYMENSLKEQEKLGIKLDKDQLIAGVQDAFADKSKLSDQEIEQTLQAFEARVKSSAQAKMEKDAADNEAKGKEYREKFAKEKGVKTSSTGLVYQVVEAGKGEAPKDSDTVVVNYKGTLIDGKEFDNSYTRGEPLSFRLDGVIPGWTEGLKNIKKGGKIKLVIPPELAYGKAGVPGIPPNSTLVFDVELLDVKPAPKADAKPEADAKAADSAKK

SEQ ID NO: 17 - DNA, 634 bp, E. Coli
tttaacatcggtaaaacctggtaagtgttctccacaaaggaatgtagtggtagtgtagcgatgactttaggcgatcaatataagatcgccgggccacgcaaagaactgcaccctccggtgcaaatgggatggtaaggagtttattgtgaaaaagtggttattagctgcaggtctcggtttagcactggcaacttctgctcaggcggctgacaaaattgcaatcgtcaacatgggcagcctgttccagcaggtagcgcagaaaaccggtgtttctaacacgctggaaaatgagttcaaaggccgtgccagcgaactgcagcgtatggaaaccgatctgcaggctaaaatgaaaaagctgcagtccatgaaagcgggcagcgatcgcactaagctggaaaaagacgtgatggctcagcgccagacttttgctcagaaagcgcaggcttttgagcaggatcgcgcacgtcgttccaacgaagaacgcggcaaactggttactcgtatccagactgctgtgaaatccgttgccaacagccaggatatcgatctggttgttgatgcaaacgccgttgcttacaacagcagcgatgtaaaagacatcactgccgacgtactgaaacaggttaaataagta

SEQ ID NO: 18 - protein, 161 aa, E. Coli
MKKWLLAAGLGLALATSAQAADKIAIVNMGSLFQQVAQKTGVSNTLENEFKGRASELQRMETDLQAKMKKLQSMKAGSDRTKLEKDVMAQRQTFAQKAQAFEQDRARRSNEERGKLVTRIQTAVKSVANSQDIDLVVDANAVAYNSSDVKDITADVLKQVK